European Patent Application EP 4 600 354 A1, published August 13, 2025. Title: PLANT CELL AND PLANT HAVING REDUCED CONTENT OF STEROIDAL GLYCOALKALOIDS AND METHODS THEREFOR. Applicant: Sveriges Stärkelseproducenter, förening upa. Application EP. The sequence listing filed with the application follows.

SEQUENCE LISTING (40 sequences)

SEQ ID NO: 1 - DNA, 24 bp, synthetic construct
  source 1..24: mol_type = other DNA
cgtcctcaagtttccaagatgtcg

SEQ ID NO: 2 - DNA, 22 bp, synthetic construct
  source 1..22: mol_type = other DNA
catcgtgttccatctggcgttg

SEQ ID NO: 3 - DNA, 20 bp, synthetic construct
  source 1..20: mol_type = other DNA
aaaggcagggtgacaccgaa

SEQ ID NO: 4 - DNA, 24 bp, synthetic construct
  source 1..24: mol_type = other DNA
gcattgctcgtacagactgttatc

SEQ ID NO: 5 - DNA, 25 bp, synthetic construct
  source 1..25: mol_type = other DNA
gccttttgagagtattgaagaggct

SEQ ID NO: 6 - DNA, 23 bp, synthetic construct
  source 1..23: mol_type = other DNA
tcataaccattggtaaagggacc

SEQ ID NO: 7 - DNA, 21 bp, synthetic construct
  source 1..21: mol_type = other DNA
gacaagtttgcccctgccatc

SEQ ID NO: 8 - DNA, 22 bp, synthetic construct
  source 1..22: mol_type = other DNA
gccaagaaaagaagctaagccc

SEQ ID NO: 9 - DNA, 21 bp, synthetic construct
  source 1..21: mol_type = other DNA
tccgagtataccgtcggagat

SEQ ID NO: 10 - DNA, 25 bp, synthetic construct
  source 1..25: mol_type = other DNA
gtgataaatgtagaagcaccagagg

SEQ ID NO: 11 - DNA, 18 bp, synthetic construct
  source 1..18: mol_type = other DNA
ccgtggtactgtgccctt

SEQ ID NO: 12 - DNA, 23 bp, synthetic construct
  source 1..23: mol_type = other DNA
gcatgcagatatttgtacagagg

SEQ ID NO: 13 - DNA, 25 bp, synthetic construct
  source 1..25: mol_type = other DNA
ttgcttcatctttctctcttgttct

SEQ ID NO: 14 - DNA, 25 bp, synthetic construct
  source 1..25: mol_type = other DNA
caaggtacttctttccatttacgtc

SEQ ID NO: 15 - DNA, 23 bp, synthetic construct
  source 1..23: mol_type = other DNA
agaagcatgggatgttggtaagt

SEQ ID NO: 16 - DNA, 24 bp, synthetic construct
  source 1..24: mol_type = other DNA
tcagtatccttcaatgctttccca

SEQ ID NO: 17 - DNA, 23 bp, synthetic construct
  source 1..23: mol_type = other DNA
ctagttaacaaaatatgtacacg

SEQ ID NO: 18 - DNA, 23 bp, synthetic construct
  source 1..23: mol_type = other DNA
gcatataacttaaaactcgtaac

SEQ ID NO: 19 - DNA, 23 bp, synthetic construct
  source 1..23: mol_type = other DNA
agaagcatgggatgttggtaagt

SEQ ID NO: 20 - DNA, 22 bp, synthetic construct
  source 1..22: mol_type = other DNA
gcagactttgtccttaactggt

SEQ ID NO: 21 - DNA, 23 bp, synthetic construct
  source 1..23: mol_type = other DNA
aactggtcaagcacattagaagc

SEQ ID NO: 22 - DNA, 24 bp, synthetic construct
  source 1..24: mol_type = other DNA
gttcttcaccattagcttttccca

SEQ ID NO: 23 - DNA, 23 bp, synthetic construct
  source 1..23: mol_type = other DNA
ggaggttattggtgcatatggag

SEQ ID NO: 24 - DNA, 23 bp, synthetic construct
  source 1..23: mol_type = other DNA
caccaatccatttgtcatccttc

SEQ ID NO: 25 - DNA, 22 bp, synthetic construct
  source 1..22: mol_type = other DNA
tgggaagccaacaattatggtg

SEQ ID NO: 26 - DNA, 20 bp, synthetic construct
  source 1..20: mol_type = other DNA
tggcaagttgtgaacagcac

SEQ ID NO: 27 - DNA, 21 bp, synthetic construct
  source 1..21: mol_type = other DNA
gctcgaaaagtactaggaggg

SEQ ID NO: 28 - DNA, 21 bp, synthetic construct
  source 1..21: mol_type = other DNA
agcaacaggttcaaaaccagc

SEQ ID NO: 29 - RNA, 20 nt, synthetic construct
  source 1..20: mol_type = other RNA
cttcctcctagggtgaacgg

SEQ ID NO: 30 - RNA, 20 nt, synthetic construct
  source 1..20: mol_type = other RNA
catcaaatggctcacccctc

SEQ ID NO: 31 - RNA, 20 nt, synthetic construct
  source 1..20: mol_type = other RNA
ctagggagaaatttgacatt

SEQ ID NO: 32 - RNA, 20 nt, synthetic construct
  source 1..20: mol_type = other RNA
ttgcagcaccttatgcccac

SEQ ID NO: 33 - RNA, 20 nt, synthetic construct
  source 1..20: mol_type = other RNA
tggctccgtaactacattgg

SEQ ID NO: 34 - RNA, 20 nt, synthetic construct
  source 1..20: mol_type = other RNA
tagtggagtttggaatctac

SEQ ID NO: 35 - RNA, 20 nt, synthetic construct
  source 1..20: mol_type = other RNA
tgcggcatggatgattgata

SEQ ID NO: 36 - RNA, 20 nt, synthetic construct
  source 1..20: mol_type = other RNA
tcaagactcaaggtgaatgg

SEQ ID NO: 37 - RNA, 20 nt, synthetic construct
  source 1..20: mol_type = other RNA
ccgatggtctttcatgcact

SEQ ID NO: 38 - RNA, 20 nt, synthetic construct
  source 1..20: mol_type = other RNA
agggtgagcaaagttatctt

SEQ ID NO: 39 - RNA, 20 nt, synthetic construct
  source 1..20: mol_type = other RNA
gatgaagaatatcttgaaag

SEQ ID NO: 40 - RNA, 20 nt, synthetic construct
  source 1..20: mol_type = other RNA
ggatggaaaatcaatgccaa